European Patent Specification EP 4 087 859 B1, published September 23, 2026. Title: PEPTIDE INTERACTING WITH TOLL-LIKE RECEPTOR 2 AND THE COMPOSITION COMPRISING THE SAME. Applicant: Chih-Hung Huang. The sequence listing filed with the application follows.

SEQUENCE LISTING (20 sequences)

SEQ ID NO: 1 - protein, 287 aa, Akkermansia muciniphila
IVNSKRSELDKKISIAAKEIKSANAAEITPSRSSNEELEKELNRYAKAVGSLETAYKPFLASSALVPTTPTAFQNELKTFRDSLISSCKKKNILITDTSSWLGFQVYSTQAPSVQAASTLGFELKAINSLVNKLAECGLSKFIKVYRPQLPIETPANNPEESDEADQAPWTPMPLEIAFQGDRESVLKAMNAITGMQDYLFTVNSIRIRNERMMPPPIANPAAAKPAAAQPATGAASLTPADEAAAPAAPAIQQVIKPYMGKEQVFVQVSLNLVHFNQPKAQEPSED

SEQ ID NO: 2 - protein, 32 aa, Akkermansia muciniphila
IVNSKRSELDKKISIAAKEIKSANAAEITPSR

SEQ ID NO: 3 - protein, 32 aa, Akkermansia muciniphila
SSNEELEKELNRYAKAVGSLETAYKPFLASSA

SEQ ID NO: 4 - protein, 27 aa, Akkermansia muciniphila
LVPTTPTAFQNELKTFRDSLISSCKKK

SEQ ID NO: 5 - protein, 34 aa, Akkermansia muciniphila
NILITDTSSWLGFQVYSTQAPSVQAASTLGFELK

SEQ ID NO: 6 - protein, 16 aa, Akkermansia muciniphila
NILITDTSSWLGFQVY

SEQ ID NO: 7 - protein, 18 aa, Akkermansia muciniphila
STQAPSVQAASTLGFELK

SEQ ID NO: 8 - protein, 25 aa, Akkermansia muciniphila
AINSLVNKLAECGLSKFIKVYRPQL

SEQ ID NO: 9 - protein, 12 aa, Akkermansia muciniphila
AINSLVNKLAEC

SEQ ID NO: 10 - protein, 13 aa, Akkermansia muciniphila
GLSKFIKVYRPQL

SEQ ID NO: 11 - protein, 24 aa, Akkermansia muciniphila
PIETPANNPEESDEADQAPWTPMP

SEQ ID NO: 12 - protein, 27 aa, Akkermansia muciniphila
LEIAFQGDRESVLKAMNAITGMQDYLF

SEQ ID NO: 13 - protein, 14 aa, Akkermansia muciniphila
LEIAFQGDRESVLK

SEQ ID NO: 14 - protein, 13 aa, Akkermansia muciniphila
AMNAITGMQDYLF

SEQ ID NO: 15 - protein, 11 aa, Akkermansia muciniphila
TVNSIRIRNER

SEQ ID NO: 16 - protein, 26 aa, Akkermansia muciniphila
MMPPPIANPAAAKPAAAQPATGAASL

SEQ ID NO: 17 - protein, 24 aa, Akkermansia muciniphila
TPADEAAAPAAPAIQQVIKPYMGK

SEQ ID NO: 18 - protein, 25 aa, Akkermansia muciniphila
EQVFVQVSLNLVHFNQPKAQEPSED

SEQ ID NO: 19 - protein, 11 aa, Akkermansia muciniphila
EQVFVQVSLNL

SEQ ID NO: 20 - protein, 14 aa, Akkermansia muciniphila
VHFNQPKAQEPSED